European Patent Application EP 4 796 567 A2, published August 26, 2026. Title: Anti-CD79 Antibodies and Their Uses. Applicant: Panorama Research Institute. Application EP. The sequence listing filed with the application follows.

SEQUENCE LISTING (77 sequences)

SEQ ID NO: 1 - protein, 119 aa, Mus musculus
QVQLQQSGPELVKPGASVKISCKASGYAFSYSWMNWVKQRPGKGLEWIGRIYPENGDTNYNGKFKGKVTLTADKSSSTAYMQLSSLTSEDSAVYFCARWVYGYPHFDYWGQGTTLTVSS

SEQ ID NO: 2 - protein, 112 aa, Mus musculus
DVVMTQTPLTLSVTIGQPASISCKSSQSLLDSDGKTYLNWLLQRPGQSPKRLIYLVSKLDSGVPDRFTGSGSGTDFTLKISRVEAEDLGVYYCWQGTHFPFTFGSGTKLEIK

SEQ ID NO: 3 - protein, 5 aa, Mus musculus
YSWMN

SEQ ID NO: 4 - protein, 17 aa, Mus musculus
RIYPENGDTNYNGKFKG

SEQ ID NO: 5 - protein, 10 aa, Mus musculus
WVYGYPHFDY

SEQ ID NO: 6 - protein, 16 aa, Mus musculus
KSSQSLLDSDGKTYLN

SEQ ID NO: 7 - protein, 7 aa, Mus musculus
LVSKLDS

SEQ ID NO: 8 - protein, 9 aa, Mus musculus
WQGTHFPFT

SEQ ID NO: 9 - protein, 119 aa, synthetic construct
QVQLVQSGAEVKKPGASVKVSCKASGYAFSYSWMNWVRQAPGQGLEWMGRIYPENGDTNYNGKFKGRVTMTRDTSISTAYMELSRLRSDDTAVYYCARWVYGYPHFDYWGQGTLVTVSS

SEQ ID NO: 10 - protein, 119 aa, synthetic construct
QVQLVQSGAEVKKPGASVKVSCKASGYAFSYSWMNWVRQAPGQGLEWMGRIYPENGDTNYNGKFKGRVTMTADTSISTAYMELSRLRSDDTAVYYCARWVYGYPHFDYWGQGTLVTVSS

SEQ ID NO: 11 - protein, 119 aa, synthetic construct
QVQLVQSGAEVKKPGASVKVSCKASGYAFSYSWMNWVRQAPGQGLEWIGRIYPENGDTNYNGKFKGRVTLTADKSISTAYMELSRLRSDDTAVYYCARWVYGYPHFDYWGQGTLVTVSS

SEQ ID NO: 12 - protein, 119 aa, synthetic construct
QVQLVQSGAEVKKPGASVKVSCKASGYAFSYSWMNWVRQAPGQGLEWMGRIYPENGDTNYAGKFKGRVTMTRDTSISTAYMELSRLRSDDTAVYYCARWVYGYPHFDYWGQGTLVTVSS

SEQ ID NO: 13 - protein, 119 aa, synthetic construct
QVQLVQSGAEVKKPGASVKVSCKASGYAFSYSWMNWVRQAPGQGLEWMGRIYPENGDTNYAGKFKGRVTMTADTSISTAYMELSRLRSDDTAVYYCARWVYGYPHFDYWGQGTLVTVSS

SEQ ID NO: 14 - protein, 119 aa, synthetic construct
QVQLVQSGAEVKKPGASVKVSCKASGYAFSYSWMNWVRQAPGQGLEWIGRIYPENGDTNYAGKFKGRVTLTADKSISTAYMELSRLRSDDTAVYYCARWVYGYPHFDYWGQGTLVTVSS

SEQ ID NO: 15 - protein, 119 aa, synthetic construct
QVQLVQSGAEVKKPGASVKVSCKASGYAFSYSWMNWVRQAPGQGLEWMGRIYPESGDTNYAGKFKGRVTMTRDTSISTAYMELSRLRSDDTAVYYCARWVYGYPHFDYWGQGTLVTVSS

SEQ ID NO: 16 - protein, 119 aa, synthetic construct
QVQLVQSGAEVKKPGASVKVSCKASGYAFSYSWMNWVRQAPGQGLEWMGRIYPESGDTNYAGKFKGRVTMTADTSISTAYMELSRLRSDDTAVYYCARWVYGYPHFDYWGQGTLVTVSS

SEQ ID NO: 17 - protein, 119 aa, synthetic construct
QVQLVQSGAEVKKPGASVKVSCKASGYAFSYSWMNWVRQAPGQGLEWIGRIYPESGDTNYAGKFKGRVTLTADKSISTAYMELSRLRSDDTAVYYCARWVYGYPHFDYWGQGTLVTVSS

SEQ ID NO: 18 - protein, 112 aa, synthetic construct
DVVMTQSPLSLPVTLGQPASISCKSSQSLLDSDGKTYLNWFQQRPGQSPRRLIYLVSKLDSGVPDRFSGSGSGTDFTLKISRVEAEDVGVYYCWQGTHFPFTFGGGTKVEIK

SEQ ID NO: 19 - protein, 112 aa, synthetic construct
DVVMTQSPLSLPVTLGQPASISCKSSQSLLDSDGKTYLNWLQQRPGQSPRRLIYLVSKLDSGVPDRFSGSGSGTDFTLKISRVEAEDVGVYYCWQGTHFPFTFGGGTKVEIK

SEQ ID NO: 20 - protein, 112 aa, synthetic construct
DVVMTQSPLSLPVTLGQPASISCKSSQSLLDSDGKTYLNWLQQRPGQSPKRLIYLVSKLDSGVPDRFSGSGSGTDFTLKISRVEAEDVGVYYCWQGTHFPFTFGGGTKVEIK

SEQ ID NO: 21 - protein, 112 aa, synthetic construct
DVVMTQSPLSLPVTLGQPASISCKSSQSLLDSSGKTYLNWFQQRPGQSPRRLIYLVSKLDSGVPDRFSGSGSGTDFTLKISRVEAEDVGVYYCWQGTHFPFTFGGGTKVEIK

SEQ ID NO: 22 - protein, 112 aa, synthetic construct
DVVMTQSPLSLPVTLGQPASISCKSSQSLLDSSGKTYLNWLQQRPGQSPRRLIYLVSKLDSGVPDRFSGSGSGTDFTLKISRVEAEDVGVYYCWQGTHFPFTFGGGTKVEIK

SEQ ID NO: 23 - protein, 112 aa, synthetic construct
DVVMTQSPLSLPVTLGQPASISCKSSQSLLDSSGKTYLNWLQQRPGQSPKRLIYLVSKLDSGVPDRFSGSGSGTDFTLKISRVEAEDVGVYYCWQGTHFPFTFGGGTKVEIK

SEQ ID NO: 24 - protein, 119 aa, unidentified
QVQLVQSGAEVKKPGASVKVSCKASGYAFSYSWMNWVRQAPGQGLEWMGRIYPENGDTNYNGKFKGRVTMTRDTSISTAYMELSRLRSDDTAVYYCARPVYGYPHFDYWGQGTLVTVSS

SEQ ID NO: 25 - protein, 119 aa, synthetic construct
QVQLVQSGAEVKKPGASVKVSCKASGYAFSYSWMNWVRQAPGQGLEWMGRIYPENGDTNYNGKFKGRVTMTRDTSISTAYMELSRLRSDDTAVYYCARWVYGLPHFDYWGQGTLVTVSS

SEQ ID NO: 26 - protein, 119 aa, synthetic construct
QVQLVQSGAEVKKPGASVKVSCKASGYAFSYSWMNWVRQAPGQGLEWMGRIYPENGDTNYNGKFKGRVTMTRDTSISTAYMELSRLRSDDTAVYYCARWVWGYPHFDYWGQGTLVTVSS

SEQ ID NO: 27 - protein, 119 aa, synthetic construct
QVQLVQSGAEVKKPGASVKVSCKASGYAFSYSWMNWVRQAPGQGLEWMGRIYPENGDTNYNGKFKGRVTMTRDTSISTAYMELSRLRSDDTAVYYCARWVYGYPHLDYWGQGTLVTVSS

SEQ ID NO: 28 - protein, 112 aa, synthetic construct
DVVMTQSPLSLPVTLGQPASISCKSSQSLLDSDGKTYLNWLQQRPGQSPRRLIYLVSKLDSGVPDRFSGSGSGTDFTLKISRVEAEDVGVYYCWQGTHIPFTFGGGTKVEIK

SEQ ID NO: 29 - protein, 112 aa, synthetic construct
DVVMTQSPLSLPVTLGQPASISCKSSQSLLDSDGKTYLNWLQQRPGQSPRRLIYLVSKLDSGVPDRFSGSGSGTDFTLKISRVEAEDVGVYYCWQGTHVPFTFGGGTKVEIK

SEQ ID NO: 30 - protein, 112 aa, synthetic construct
DVVMTQSPLSLPVTLGQPASISCKSSQSLLDSDGKTYLNWLQQRPGQSPRRLIYLVSKLDSGVPDRFSGSGSGTDFTLKISRVEAEDVGVYYCWQGTHLPFTFGGGTKVEIK

SEQ ID NO: 31 - protein, 112 aa, synthetic construct
DVVMTQSPLSLPVTLGQPASISCKSSQSLLDSDGKTYLNWLQQRPGQSPRRLIYLVSKLDSGVPDRFSGSGSGTDFTLKISRVEAEDVGVYYCWQGTHRPFTFGGGTKVEIK

SEQ ID NO: 32 - protein, 119 aa, synthetic construct
QVQLVQSGAEVKKPGASVKVSCKASGYAFSYSWINWVRQAPGQGLEWMGRIYPENGDTNYNGKFKGRVTMTRDTSISTAYMELSRLRSDDTAVYYCARWVYGYPHFDYWGQGTLVTVSS

SEQ ID NO: 33 - protein, 119 aa, synthetic construct
QVQLVQSGAEVKKPGASVKVSCKASGYAFGYSWMNWVRQAPGQGLEWMGRIYPENGDTNYNGKFKGRVTMTRDTSISTAYMELSRLRSDDTAVYYCARWVYGYPHFDYWGQGTLVTVSS

SEQ ID NO: 34 - protein, 119 aa, synthetic construct
QVQLVQSGAEVKKPGASVKVSCKASGYAFSYSWMNWVRQAPGQGLEWMGRIYPENGDTNYNGKFKGRVTMTRDTSISTAYMELSRLRPDDTAVYYCARWVYGYPHFDYWGQGTLVTVSS

SEQ ID NO: 35 - protein, 119 aa, synthetic construct
QVQLVQSGAEVKKPGASVKVSCKASGYAFNYSWMNWVRQVPGQGLEWMGRIYPENGDTNYNGKFKGRVTMTRDTSISTAYMELSRLRSDDTAVYYCARWVYGYPHFDYWGQGTLVTVSS

SEQ ID NO: 36 - protein, 119 aa, synthetic construct
QVQLVQSGAEVKKPGASVKVSCKASGYAFSYSWMNWVRQAPGQGLEWMGRIYPENGDTNYNGKFKGRVTMTRDTSINTAYMELSRLRSDDTAVYYCARWVYGYPHFDYWGQGTLVTVSS

SEQ ID NO: 37 - protein, 119 aa, synthetic construct
QVQLVQSGAEVKKPGASVKVSCKASGYAFSYSWVNWVRQAPGQGLEWMGRIYPENGDTNYNGKFKGRVTMTRDTSISTAYMELSRLRSDDTAVYYCARWVYGYPHFDYWGQGTLVTVSS

SEQ ID NO: 38 - protein, 119 aa, synthetic construct
QVQLVQSGAEVKKPGASVKVSCKASGYAFSYSWMNWVRQAPGQGLEWMGRIYPENGDTNYNGKFKGRVTMTRDTSISTAYMELSGLRSDDTAVYYCARWVYGYPHFDYWGQGTLVTVSS

SEQ ID NO: 39 - protein, 119 aa, synthetic construct
QVQLVQSGAEVKKPGASVKVSCKASGYAFNYSWVNWVRQAPGQGFEWMGRIYPENGDTNYNGKFKGRVTMTRDTSISTAYMELSRLRSDDTAVYYCARWVYGYPHFDYWGQGTLVTVSS

SEQ ID NO: 40 - protein, 119 aa, synthetic construct
QVQLVQSGAEVKKPGASVKVSCKASGYAFRYSWMNWVRQAPGQGLEWMGRIYPENGGTNYNGKFKGRVTMTMDTSISTAYMELSRLRSDDTAVYYCARWVYGYPHFDYWGQGTLVTVSS

SEQ ID NO: 41 - protein, 119 aa, synthetic construct
QVQLVQSGAEVKKPGASVKVSCKASGYAFSYSWMNWVRQAPGQGLEWMGRIYPENGDTNYNGKFRGRVTMTRDTSISTAYMELSRLRSDDTAVYYCARWVYGYPHFDYWGQGTLVTVSS

SEQ ID NO: 42 - protein, 112 aa, synthetic construct
DVVMTQSPLSLPVTLGLPASISCKSSQSLLDSDGKTYLNWLQQRPGQSPRRLIYLVSKLDSGVPDRFSGSGSGTDFTLKISRVEAEDVGVYYCWQGTHFPFTFGGGTKVEIK

SEQ ID NO: 43 - protein, 112 aa, synthetic construct
DVVMTQSPLSLPVTLGQPASISCKSSKSLLDSDGKTYLNWLQQRPGQSPRRLIYLVSKLDSGVPDRFSGSGSGTDFTLKISRVEAEDVGVYYCWQGTHFPFTFGGGTKVEIK

SEQ ID NO: 44 - protein, 112 aa, synthetic construct
DVVMTQSPLSLPVTLGQPASISCKSSQSLLDSDGKTYLNWLQQRPGQSPRRIIYLVSKLDSGVPDRFSGSGSGTDFTLKISRVEAEDVGVYYCWQGTHFPFTFGGGTKVEIK

SEQ ID NO: 45 - protein, 112 aa, synthetic construct
DVVMTQSPLSLPVTLGQPASISCKSSQSLLDSDGKTYLNWLQQRPGQSPRRLIYLVSKLDSGVPDRFSGSGSGTDFTLKISRVEADDVGVYYCWQGTHLPFTFGGGTKVEIK

SEQ ID NO: 46 - protein, 112 aa, synthetic construct
DVVMTQSPLSLPVTLGQPASISCKSSQSLLDSDGKTYLNWLQQRPGQSPRRLIYLVSKLDSGVPDRFSGSGSGTDFTLKISRVEAEDVGFYYCWQGTHLPFTFGGGTKVEIK

SEQ ID NO: 47 - protein, 112 aa, synthetic construct
DVVMTQSPLSLPVTLGQTASISCKSSQSLLDSDGKTYLNWLQQRPGQSPRRLIYLVSKLDSGVPDRFSGSGSGTDFTLKISRVEAEDVGVYYCWQGTHLPFTFGGGTKVEIK

SEQ ID NO: 48 - protein, 112 aa, synthetic construct
DVVMTQSPLSLPVTLGRPASISCKSSQSLLDSGGKTYLNWLQQRPGQSPRRLIYLVSKLDSGVPDRFSGSGSGTDFTLKISRVEAEDVGVYYCWQGTHFPFTFGGGTKVEIK

SEQ ID NO: 49 - protein, 112 aa, synthetic construct
DVVMTQSPLSLPVTLGQPASISCKSSRSLLDSDGKTYLNWLQQRPGQSPRRLIYLVSKLDSGVPDRFSGSGSGTDFTLKISRVEAEDVGVYYCWQGTHFPFTFGGGTKVEIK

SEQ ID NO: 50 - protein, 112 aa, synthetic construct
DVVMTQSPLSLPVTLGLPASISCKSSQSLLDTDGKTYLNWLQQRPGQSPRRLIYLVSKLDSGVPDRFIGSGSGTDFTLKISRVEAEDVGVYYCWQGTHFPFTFGGGTKVEIK

SEQ ID NO: 51 - protein, 112 aa, synthetic construct
DVVMTQSPLSLPVTLGQPASISCKSSQSLLDSDGKTYLNWLQQRPGQPPRRLIYLVSKLDSGVPDRFSGSGSGTDFTLKISRVEAEDVGVYYCWQGTHFPFTFGGGTKVEIK

SEQ ID NO: 52 - protein, 112 aa, synthetic construct
DVVMTQSPLSLPVTLGQPASITCKSSQSLLDSDGKTYLNWLQQRPGQSPRRLIYLVSKPDSGVPDRFSGSGSGTDFTLKISRVEAEDVGVYYCWQGTHFPFTFGGGTKVEIK

SEQ ID NO: 53 - protein, 112 aa, synthetic construct
DVVMTQSPPSLPVTLGQPASISCKSSQSLLDSDGKTYLNWLQQRPGQSPRRLIYLVSKLDSGVPDRFSGSGSGTDFTLKISRVEAEDVGVYYCWQGTHVPFTFGGGTKVEIK

SEQ ID NO: 54 - protein, 112 aa, synthetic construct
DVVMTQSPLSLPVTLGQTASISCKSSQSLLDRDGKTYLNWLQQRPGQSPRRIIYLVSKLDSGVPDRFSGSGSGTDFTLKISRVEAEDVGVYYCWQGTHFPFTFGGGTKVEIK

SEQ ID NO: 55 - protein, 112 aa, synthetic construct
DVVMTQSPLSMPVTLGLPASISCKSSQSLLDSHGKTYLNWLQQRPGQSPRRLIYLVSKLDSGVPDRFSGSGSGTDFTLKISRVEAEDVGVYYCWQGTHFPFTFGGGTKVEIK

SEQ ID NO: 56 - protein, 112 aa, synthetic construct
DVVMTQSPLSLPVTLGLPASISCKSSQSLLDSDGKTYLNWLQQRPGQSPRRLIYLVSKLDSGVPDRFSGSGSGTDFTLKISRVEAEDVGVYYCWQGTHIPFTFSGGTKVEIK

SEQ ID NO: 57 - protein, 16 aa, synthetic construct
KSSQSLLDSSGKTYLN

SEQ ID NO: 58 - protein, 17 aa, synthetic construct
RIYPENGDTNYAGKFKG

SEQ ID NO: 59 - protein, 17 aa, synthetic construct
RIYPESGDTNYAGKFKG

SEQ ID NO: 60 - protein, 15 aa, synthetic construct
WFQQRPGQSPRRLIY

SEQ ID NO: 61 - protein, 15 aa, synthetic construct
WLQQRPGQSPRRLIY

SEQ ID NO: 62 - protein, 15 aa, synthetic construct
WLQQRPGQSPKRLIY

SEQ ID NO: 63 - protein, 30 aa, synthetic construct
QVQLVQSGAEVKKPGASVKVSCKASGYAFS

SEQ ID NO: 64 - protein, 14 aa, synthetic construct
WVRQAPGQGLEWMG

SEQ ID NO: 65 - protein, 32 aa, synthetic construct
RVTMTRDTSISTAYMELSRLRSDDTAVYYCAR

SEQ ID NO: 66 - protein, 32 aa, synthetic construct
RVTMTADTSISTAYMELSRLRSDDTAVYYCAR

SEQ ID NO: 67 - protein, 14 aa, synthetic construct
WVRQAPGQGLEWIG

SEQ ID NO: 68 - protein, 32 aa, synthetic construct
RVTLTADKSISTAYMELSRLRSDDTAVYYCAR

SEQ ID NO: 69 - DNA, 1415 bp, synthetic construct
  source 1..1415: mol_type = other DNA
gatgttgtgatgactcagtctccactctccctgcccgtcacccttggacagccggcctccatctcctgcaagtcaagtcagagcctcttagatagtgatggaaagacatatttgaattggttacagcagaggccaggccaatctccaaggcgcctaatttatctggtgtctaaactggactctggggtcccagacagattcagcggcagtgggtcaggcactgatttcacactgaaaatcagcagggtggaagctgaggatgttggggtttattactgctggcaaggtacacatctgccattcacgttcggcggagggaccaaggtggagatcaaaggtggcggtggctcgggcggtggtgggtcgggtggcggcggatctcaggtgcagctggtgcagtctggggctgaggtgaagaagcctggggcctcagtgaaggtctcctgcaaggcttctggatacgcattcagttactcctggatgaactgggtgcgacaggcccctggacaagggcttgagtggatgggacggatttatcctgaaaatggagatactaactacaatgggaagttcaagggcagggtcaccatgaccagggacacgtccatcagcacagcctacatggagctgagcaggctgagatctgacgacacggccgtgtattactgtgcgagatgggtctatggtcttccccactttgactactggggccaaggaaccctggtcaccgtctcctcagctagcaccacgacgccagcgccgcgaccaccaacaccggcgcccaccatcgcgtcgcagcccctgtccctgcgcccagaggcgtgccggccagcggcggggggcgcagtgcacacgagggggctggacttcgcctgtgatatctacatctgggcgcccttggccgggacttgtggggtccttctcctgtcactggttatcaccctttactgcaaacggggcagaaagaaactcctgtatatattcaaacaaccatttatgagaccagtacaaactactcaagaggaagatggctgtagctgccgatttccagaagaagaagaaggaggatgtgaactgagagtgaagttcagcaggagcgcagacgccccgcgtacaagcagggccagaaccagctctataacgagctcaatctaggacgaagagaggagtacgatgttttggacaagagacgtggccgggaccctgagatggggggaaagccgagaaggaagaacccccaggaaggcctgtacaatgaactgcagaaagataagatggcggaggcctacagtgagattgggatgaaaggcgagcgccggaggggcaaggggcacgatggcctttaccagggtctcagtacagccaccaaggacacctacgacgcccttcacatgcaggccctgccccctcgctga

SEQ ID NO: 70 - protein, 470 aa, synthetic construct
DVVMTQSPLSLPVTLGQPASISCKSSQSLLDSDGKTYLNWLQQRPGQSPRRLIYLVSKLDSGVPDRFSGSGSGTDFTLKSRVEAEDVGVYYCWQGTHLPFTFGGGTKVEIKGGGGSGGGGSGGGGSQVQLVQSGAEVKKPGASVKVSCKASGYAFSYSWMNWVRQAPGQGLEWMGRIYPENGDTNYNGKFKGRVTMTRDTSISTAYMELSRLRSDDTAVYYCARWVYGLPHFDYWGQGTLVTVSSASTTTPAPRPPTPAPTIASQPLSLRPEACRPAAGGAVHTRGLDFACDIYIWAPLAGTCGVLLLSLVITLYCKRGRKKLLYIFKQPFMRPVQTTQEEDGCSCRFPEEEEGGCELRVKFSRSADAPAYKQGQNQLYNELNLGRREEYDVLDKRRGRDPEMGGKPRRKNPQEGLYNELQKDKMAEAYSEIGMKGERRRGKGHDGLYQGLSTATKDTYDALHMQALPPR

SEQ ID NO: 71 - protein, 119 aa, synthetic construct; identical to SEQ ID NO: 39

SEQ ID NO: 72 - protein, 119 aa, synthetic construct; identical to SEQ ID NO: 39

SEQ ID NO: 73 - protein, 112 aa, synthetic construct; identical to SEQ ID NO: 30

SEQ ID NO: 74 - protein, 112 aa, synthetic construct; identical to SEQ ID NO: 30

SEQ ID NO: 75 - protein, 119 aa, synthetic construct
QVQLVQSGAEVKKPGASVKVSCKASGYAFSYSWMNWVRQAPGQGLEWMGRIYPESGDTNYNGKFKGRVTMTRDTSISTAYMELSRLRSDDTAVYYCARWVYGLPHFDYWGQGTLVTVSS

SEQ ID NO: 76 - protein, 119 aa, synthetic construct
QVQLVQSGAEVKKPGASVKVSCKASGYAFSYSWMNWVRQAPGQGLEWMGRIYPENGDTNYAGKFKGRVTMTRDTSISTAYMELSRLRSDDTAVYYCARWVYGLPHFDYWGQGTLVTVSS

SEQ ID NO: 77 - protein, 119 aa, synthetic construct
QVQLVQSGAEVKKPGASVKVSCKASGYAFSYSWMNWVRQAPGQGLEWMGRIYPESGDTNYAGKFKGRVTMTRDTSISTAYMELSRLRSDDTAVYYCARWVYGLPHFDYWGQGTLVTVSS